European Patent Application EP 4 778 936 A1, published July 22, 2026. Title: Variant of twin-arginine translocase and method for producing target protein using the same. Applicant: CJ CheilJedang Corporation. The sequence listing filed with the application follows.

SEQUENCE LISTING (75 sequences)

SEQ ID NO: 1 - protein, 314 aa, synthetic construct
  REGION 1..314: note = TatC protein derived from Corynebactrium glutamicum ATCC13032 (WP_011014400.1)
MSIVEHIKEFRRRLLIALAGILVGTIIGFIWYDFSFWQIPTLGELLRDPYCSLPAESRWAMSDSEECRLLATGPFDPFMLRLKVAALVGMVLGSPVWLSQLWGFITPGLMKNERRYTAIFVTIAVVLFVGGAVLAYFVVAYGLEFLLTIGGDTQAAALTGDKYFGFLLALLAIFGVSFEVPLVIGMLNIVGILPYDAIKDKRRMIIMILFVFAAFMTPGQDPFTMLVLALSLTVLVELALQFCRFNDKRRDKKRPEWLDGDDLSASPLDTSAGGEDAPSPVETPEAVEPSRMLNPSGEASISYKPGRADFGDVL

SEQ ID NO: 2 - DNA, 945 bp, synthetic construct
  misc_feature 1..945: note = gene coding TatC protein derived from Corynebactrium glutamicum ATCC13032
  source 1..945: mol_type = other DNA
atgtccattgttgagcacatcaaagagtttcgacgccgacttcttatcgctctggcgggcatcctcgtgggcaccattatcggctttatttggtacgatttctcattttggcagatccccactttgggcgagctgctgagggatccgtactgttctctgcctgctgaatcccgctgggccatgagcgactcagaggaatgtcgactgctcgcaaccggcccgtttgatccattcatgcttcgccttaaagtagcggcgttggtgggtatggttcttggctcacccgtgtggctgagccagctgtggggctttatcaccccaggtttgatgaagaatgagcgccgttacaccgcaatcttcgtcacgattgctgttgtgctgtttgtcggcggtgctgttcttgcgtacttcgtcgttgcatatggtttggagttcctccttaccattggtggagacacccaggcagcggccctgactggtgataagtacttcggattcttgctcgcgttgttggcgattttcggcgtgagcttcgaagttccactggtgatcggcatgctcaacattgtgggtatcttgccttacgatgccattaaagataagcgacgcatgatcatcatgattttgttcgtgttcgctgctttcatgacacccggccaggatcctttcaccatgttggtgttggcgctttcactcaccgttctggtagagcttgccctgcagttctgtcgtttcaacgacaaacgccgggacaagaagcgcccagaatggcttgatggcgatgacctctctgcatcaccactggatacttctgctggtggagaagatgctccaagcccagtcgaaaccccagaggcggtggagccttcgcggatgctgaacccaagtggggaggcgtcgataagctataaacccgggcgcgccgacttcggtgacgtgctctaa

SEQ ID NO: 3 - protein, 258 aa, synthetic construct
  REGION 1..258: note = TatC protein derived from Escherichia coli K-12 (WP_000109943.1)
MSVEDTQPLITHLIELRKRLLNCIIAVIVIFLCLVYFANDIYHLVSAPLIKQLPQGSTMIATDVASPFFTPIKLTFMVSLILSAPVILYQVWAFIAPALYKHERRLVVPLLVSSSLLFYIGMAFAYFVVFPLAFGFLANTAPEGVQVSTDIASYLSFVMALFMAFGVSFEVPVAIVLLCWMGITSPEDLRKKRPYVLVGAFVVGMLLTPPDVFSQTLLAIPMYCLFEIGVFFSRFYVGKGRNREEENDAEAESEKTEE

SEQ ID NO: 4 - DNA, 777 bp, synthetic construct
  misc_feature 1..777: note = gene coding TatC protein derived from Escherichia coli K-12
  source 1..777: mol_type = other DNA
atgtctgtagaagatactcaaccgcttatcacgcatctgattgagctgcgtaagcgtctgctgaactgcattatcgcggtgatcgtgatattcctgtgtctggtctatttcgccaatgacatctatcacctggtatccgcgccattgatcaagcagttgccgcaaggttcaacgatgatcgccaccgacgtggcctcgccgttctttacgccgatcaagctgacctttatggtgtcgctgattctgtcagcgccggtgattctctatcaggtgtgggcatttatcgccccagcgctgtataagcatgaacgtcgcctggtggtgccgctgctggtttccagctctctgctgttttatatcggcatggcattcgcctactttgtggtctttccgctggcatttggcttccttgccaataccgcgccggaaggggtgcaggtatccaccgacatcgccagctatttaagcttcgttatggcgctgtttatggcgtttggtgtctcctttgaagtgccggtagcaattgtgctgctgtgctggatggggattacctcgccagaagacttacgcaaaaaacgcccgtatgtgctggttggtgcattcgttgtcgggatgttgctgacgccgccggatgtcttctcgcaaacgctgttggcgatcccgatgtactgtctgtttgaaatcggtgtcttcttctcacgcttttacgttggtaaagggcgaaatcgggaagaggaaaacgacgctgaagcagaaagcgaaaaaactgaagaataa

SEQ ID NO: 5 - protein, 1027 aa, synthetic construct
  REGION 1..1027: note = bovine COL6A1 (NP_001137337.1)
MRLPRALLPLLLQACWASAQDDPVASRAIAFQDCPVDLFFVLDTSESVALRLKPYGALVDKVKSFTKRFIDNLNDRYYRCDRNLVWNAGALHYSDEVEIIRGLTRMPSGRDELKSSVDAVKYFGKGTYTDCAIKKGLEELLVGGSHLKENKYLVVVTDGHPLEGYKEPCGGLEDAVNEAKHLGIKVFSVAITPDHLEPRLSIIATDHTYRRNFTAADWGQSRDAEEVISQTIDTITDMIKNNVEQVCCSFECQPARGPPGPRGDPGYEGERGKPGLPGEKGEAGDPGRPGDLGPVGYQGMKGEKGSRGEKGSRGPKGYKGEKGKRGMDGVDGMKGETGFPGLPGCKGSPGFDGIQGPPGPKGDPGAFGLKGQKGEPGADGEPGRPGSTGPPGDEGEPGEPGPPGEKGEAGDEGNAGPDGAPGERGGPGERGPRGTPGARGPRGDPGEAGPQGDQGREGPVGVPGDPGEAGPIGPKGYRGDEGPPGTEGPKGAPGPAGPPGDPGLMGERGEDGPPGNGTEGFPGFPGYPGSRGPPGINGTKGYPGLKGDEGEAGDPGEDNNDIAARGAKGAKGYRGPEGPQGPPGHVGPPGPDECEILDIIMKMCSCCECKCGPIDILFVLDSSESIGLQNFEIAKDFIVKVIDRLSKDELVKFEPGQSHAGVVQYSHNQMQEHVDLRDPNIRNAQDLKEAIKKLQWMGGGTFTGEALQYTRSRLLPPTPNNRIALVITDGRSDTQRDTTPLSVLCGPDIQVVSVGIKDVFGLAAGSDQLNVISCQGLAPQGRPGISLVKENYAELLDDGFLKNITAQICIDKKCPDYSCPITFSSPADITILLDGSASVGSHNFDITKRFAKRLAERFLTASRTDPGQDVRVAVVQYSGTGQQRPERAALQFLQNYTVLANTVDSMDFFNDATDVMDALGYVTRFYREASSNAAKKRLLLFSDGNSQGATPAAIEKAVQEAQRAGVEIFAVVVGRQVNEPHVRVLVTGKAAEYDVVFGERHLFRVPSYQALLRGVFYQTVSRKVALD

SEQ ID NO: 6 - protein, 106 aa, synthetic construct
  REGION 1..106: note = bCOL6_1 polypeptide
GGPGERGPRGTPGARGPRGDPGEAGPQGDQGREGPVGVPGDPGEAGPIGPKGYRGDEGPPGTEGPKGAPGPAGPPGDPGLMGERGEDGPPGNGTEGFPGFHHHHHH

SEQ ID NO: 7 - DNA, 321 bp, synthetic construct
  misc_feature 1..321: note = gene coding bCOL6_1 polypeptide
  source 1..321: mol_type = other DNA
ggtggacctggtgaacggggcccacggggtactcctggggcgcgtggaccgagaggtgatcctggcgaagccgggcctcagggggatcaggggcgcgagggaccagtcggagttccaggggacccaggggaggccggaccgataggccctaaaggataccgcggtgacgaaggtccgcccggaacagaaggacctaaaggggcccccggacccgctggtcctccaggggatccagggctgatgggtgagcgtggtgaagatggtcctcccggcaacggtacggaaggctttcctggctttcatcaccatcaccatcactaa

SEQ ID NO: 8 - protein, 33 aa, synthetic construct
  REGION 1..33: note = CgR0949 signal peptide
MQINRRGFLKATTGLATIGAASMFMPKANALGA

SEQ ID NO: 9 - DNA, 99 bp, synthetic construct
  misc_feature 1..99: note = gene coding CgR0949 signal peptide
  source 1..99: mol_type = other DNA
atgcaaataaaccgccgaggcttcttaaaagccaccacaggacttgccactatcggcgctgccagcatgtttatgccaaaggccaacgcccttggagca

SEQ ID NO: 10 - DNA, 318 bp, synthetic construct
  misc_feature 1..318: note = cj7 protomer
  source 1..318: mol_type = other DNA
agaaacatcccagcgctactaatagggagcgttgaccttccttccacggaccggtaatcggagtgcctaaaaccgcatgcggcttaggctccaagataggttctgcgcggccgggtaatgcatcttctttagcaacaagttgaggggtaggtgcaaataagaacgacatagaaatcgtctcctttctgtttttaatcaacatacaccaccacctaaaaattccccgaccagcaagttcacagtattcgggcacaatatcgttgccaaaatattgtttcggaatatcatgggatacgtacccaacgaaaggaaacactc

SEQ ID NO: 11 - DNA, 364 bp, synthetic construct
  misc_feature 1..364: note = pyk promoter
  source 1..364: mol_type = other DNA
tcgtgttcttcctgttgaagaagggtagggaaactcccgaagaggtagatccgactttcgcagcgtctgttgcagcagatgctgtagcttcgccggatggaaaacccttgccgaaagcaggggagggcattgatggagaaacgccctcaacgcgataggtttcaaccataggcctgacctggctgagatgtttttggtagaaaaaccgagtgcccgaattgttttgtgggtgcccggttttttctgatttaagcacgtcagaggcgtagaacattgtctgttcacactctgggtcgcaagattcatcgagaattaatggtagtacctgtggcttgagggggaatgacgtactaggcttatgggc

SEQ ID NO: 12 - protein, 314 aa, synthetic construct
  REGION 1..314: note = TatC T106A variant, wherein the TatC is derived from Corynebactrium glutamicum ATCC13032
MSIVEHIKEFRRRLLIALAGILVGTIIGFIWYDFSFWQIPTLGELLRDPYCSLPAESRWAMSDSEECRLLATGPFDPFMLRLKVAALVGMVLGSPVWLSQLWGFIAPGLMKNERRYTAIFVTIAVVLFVGGAVLAYFVVAYGLEFLLTIGGDTQAAALTGDKYFGFLLALLAIFGVSFEVPLVIGMLNIVGILPYDAIKDKRRMIIMILFVFAAFMTPGQDPFTMLVLALSLTVLVELALQFCRFNDKRRDKKRPEWLDGDDLSASPLDTSAGGEDAPSPVETPEAVEPSRMLNPSGEASISYKPGRADFGDVL

SEQ ID NO: 13 - DNA, 945 bp, synthetic construct
  misc_feature 1..945: note = gene coding TatC T106A variant, wherein the TatC is derived from Corynebactrium glutamicum ATCC13032
  source 1..945: mol_type = other DNA
atgtccattgttgagcacatcaaagagtttcgacgccgacttcttatcgctctggcgggcatcctcgtgggcaccattatcggctttatttggtacgatttctcattttggcagatccccactttgggcgagctgctgagggatccgtactgttctctgcctgctgaatcccgctgggccatgagcgactcagaggaatgtcgactgctcgcaaccggcccgtttgatccattcatgcttcgccttaaagtagcggcgttggtgggtatggttcttggctcacccgtgtggctgagccagctgtggggctttatcgcaccaggtttgatgaagaatgagcgccgttacaccgcaatcttcgtcacgattgctgttgtgctgtttgtcggcggtgctgttcttgcgtacttcgtcgttgcatatggtttggagttcctccttaccattggtggagacacccaggcagcggccctgactggtgataagtacttcggattcttgctcgcgttgttggcgattttcggcgtgagcttcgaagttccactggtgatcggcatgctcaacattgtgggtatcttgccttacgatgccattaaagataagcgacgcatgatcatcatgattttgttcgtgttcgctgctttcatgacacccggccaggatcctttcaccatgttggtgttggcgctttcactcaccgttctggtagagcttgccctgcagttctgtcgtttcaacgacaaacgccgggacaagaagcgcccagaatggcttgatggcgatgacctctctgcatcaccactggatacttctgctggtggagaagatgctccaagcccagtcgaaaccccagaggcggtggagccttcgcggatgctgaacccaagtggggaggcgtcgataagctataaacccgggcgcgccgacttcggtgacgtgctctaa

SEQ ID NO: 14 - protein, 314 aa, synthetic construct
  REGION 1..314: note = TatC P107S variant, wherein the TatC is derived from Corynebactrium glutamicum ATCC13032
MSIVEHIKEFRRRLLIALAGILVGTIIGFIWYDFSFWQIPTLGELLRDPYCSLPAESRWAMSDSEECRLLATGPFDPFMLRLKVAALVGMVLGSPVWLSQLWGFITSGLMKNERRYTAIFVTIAVVLFVGGAVLAYFVVAYGLEFLLTIGGDTQAAALTGDKYFGFLLALLAIFGVSFEVPLVIGMLNIVGILPYDAIKDKRRMIIMILFVFAAFMTPGQDPFTMLVLALSLTVLVELALQFCRFNDKRRDKKRPEWLDGDDLSASPLDTSAGGEDAPSPVETPEAVEPSRMLNPSGEASISYKPGRADFGDVL

SEQ ID NO: 15 - DNA, 945 bp, synthetic construct
  misc_feature 1..945: note = gene coding TatC P107S variant, wherein the TatC is derived from Corynebactrium glutamicum ATCC13032
  source 1..945: mol_type = other DNA
atgtccattgttgagcacatcaaagagtttcgacgccgacttcttatcgctctggcgggcatcctcgtgggcaccattatcggctttatttggtacgatttctcattttggcagatccccactttgggcgagctgctgagggatccgtactgttctctgcctgctgaatcccgctgggccatgagcgactcagaggaatgtcgactgctcgcaaccggcccgtttgatccattcatgcttcgccttaaagtagcggcgttggtgggtatggttcttggctcacccgtgtggctgagccagctgtggggctttatcacctccggtttgatgaagaatgagcgccgttacaccgcaatcttcgtcacgattgctgttgtgctgtttgtcggcggtgctgttcttgcgtacttcgtcgttgcatatggtttggagttcctccttaccattggtggagacacccaggcagcggccctgactggtgataagtacttcggattcttgctcgcgttgttggcgattttcggcgtgagcttcgaagttccactggtgatcggcatgctcaacattgtgggtatcttgccttacgatgccattaaagataagcgacgcatgatcatcatgattttgttcgtgttcgctgctttcatgacacccggccaggatcctttcaccatgttggtgttggcgctttcactcaccgttctggtagagcttgccctgcagttctgtcgtttcaacgacaaacgccgggacaagaagcgcccagaatggcttgatggcgatgacctctctgcatcaccactggatacttctgctggtggagaagatgctccaagcccagtcgaaaccccagaggcggtggagccttcgcggatgctgaacccaagtggggaggcgtcgataagctataaacccgggcgcgccgacttcggtgacgtgctctaa

SEQ ID NO: 16 - protein, 314 aa, synthetic construct
  REGION 1..314: note = TatC G108A variant, wherein the TatC is derived from Corynebactrium glutamicum ATCC13032
MSIVEHIKEFRRRLLIALAGILVGTIIGFIWYDFSFWQIPTLGELLRDPYCSLPAESRWAMSDSEECRLLATGPFDPFMLRLKVAALVGMVLGSPVWLSQLWGFITPALMKNERRYTAIFVTIAVVLFVGGAVLAYFVVAYGLEFLLTIGGDTQAAALTGDKYFGFLLALLAIFGVSFEVPLVIGMLNIVGILPYDAIKDKRRMIIMILFVFAAFMTPGQDPFTMLVLALSLTVLVELALQFCRFNDKRRDKKRPEWLDGDDLSASPLDTSAGGEDAPSPVETPEAVEPSRMLNPSGEASISYKPGRADFGDVL

SEQ ID NO: 17 - DNA, 945 bp, synthetic construct
  misc_feature 1..945: note = gene coding TatC G108A variant, wherein the TatC is derived from Corynebactrium glutamicum ATCC13032
  source 1..945: mol_type = other DNA
atgtccattgttgagcacatcaaagagtttcgacgccgacttcttatcgctctggcgggcatcctcgtgggcaccattatcggctttatttggtacgatttctcattttggcagatccccactttgggcgagctgctgagggatccgtactgttctctgcctgctgaatcccgctgggccatgagcgactcagaggaatgtcgactgctcgcaaccggcccgtttgatccattcatgcttcgccttaaagtagcggcgttggtgggtatggttcttggctcacccgtgtggctgagccagctgtggggctttatcaccccagcattgatgaagaatgagcgccgttacaccgcaatcttcgtcacgattgctgttgtgctgtttgtcggcggtgctgttcttgcgtacttcgtcgttgcatatggtttggagttcctccttaccattggtggagacacccaggcagcggccctgactggtgataagtacttcggattcttgctcgcgttgttggcgattttcggcgtgagcttcgaagttccactggtgatcggcatgctcaacattgtgggtatcttgccttacgatgccattaaagataagcgacgcatgatcatcatgattttgttcgtgttcgctgctttcatgacacccggccaggatcctttcaccatgttggtgttggcgctttcactcaccgttctggtagagcttgccctgcagttctgtcgtttcaacgacaaacgccgggacaagaagcgcccagaatggcttgatggcgatgacctctctgcatcaccactggatacttctgctggtggagaagatgctccaagcccagtcgaaaccccagaggcggtggagccttcgcggatgctgaacccaagtggggaggcgtcgataagctataaacccgggcgcgccgacttcggtgacgtgctctaa

SEQ ID NO: 18 - protein, 314 aa, synthetic construct
  REGION 1..314: note = TatC T106A/P107S variant, wherein the TatC is derived from Corynebactrium glutamicum ATCC13032
MSIVEHIKEFRRRLLIALAGILVGTIIGFIWYDFSFWQIPTLGELLRDPYCSLPAESRWAMSDSEECRLLATGPFDPFMLRLKVAALVGMVLGSPVWLSQLWGFIASGLMKNERRYTAIFVTIAVVLFVGGAVLAYFVVAYGLEFLLTIGGDTQAAALTGDKYFGFLLALLAIFGVSFEVPLVIGMLNIVGILPYDAIKDKRRMIIMILFVFAAFMTPGQDPFTMLVLALSLTVLVELALQFCRFNDKRRDKKRPEWLDGDDLSASPLDTSAGGEDAPSPVETPEAVEPSRMLNPSGEASISYKPGRADFGDVL

SEQ ID NO: 19 - DNA, 945 bp, synthetic construct
  misc_feature 1..945: note = gene coding TatC T106A/P107S variant, wherein the TatC is derived from Corynebactrium glutamicum ATCC13032
  source 1..945: mol_type = other DNA
atgtccattgttgagcacatcaaagagtttcgacgccgacttcttatcgctctggcgggcatcctcgtgggcaccattatcggctttatttggtacgatttctcattttggcagatccccactttgggcgagctgctgagggatccgtactgttctctgcctgctgaatcccgctgggccatgagcgactcagaggaatgtcgactgctcgcaaccggcccgtttgatccattcatgcttcgccttaaagtagcggcgttggtgggtatggttcttggctcacccgtgtggctgagccagctgtggggctttatcgcatccggtttgatgaagaatgagcgccgttacaccgcaatcttcgtcacgattgctgttgtgctgtttgtcggcggtgctgttcttgcgtacttcgtcgttgcatatggtttggagttcctccttaccattggtggagacacccaggcagcggccctgactggtgataagtacttcggattcttgctcgcgttgttggcgattttcggcgtgagcttcgaagttccactggtgatcggcatgctcaacattgtgggtatcttgccttacgatgccattaaagataagcgacgcatgatcatcatgattttgttcgtgttcgctgctttcatgacacccggccaggatcctttcaccatgttggtgttggcgctttcactcaccgttctggtagagcttgccctgcagttctgtcgtttcaacgacaaacgccgggacaagaagcgcccagaatggcttgatggcgatgacctctctgcatcaccactggatacttctgctggtggagaagatgctccaagcccagtcgaaaccccagaggcggtggagccttcgcggatgctgaacccaagtggggaggcgtcgataagctataaacccgggcgcgccgacttcggtgacgtgctctaa

SEQ ID NO: 20 - protein, 314 aa, synthetic construct
  REGION 1..314: note = TatC P107S/G108A variant, wherein the TatC is derived from Corynebactrium glutamicum ATCC13032
MSIVEHIKEFRRRLLIALAGILVGTIIGFIWYDFSFWQIPTLGELLRDPYCSLPAESRWAMSDSEECRLLATGPFDPFMLRLKVAALVGMVLGSPVWLSQLWGFITSALMKNERRYTAIFVTIAVVLFVGGAVLAYFVVAYGLEFLLTIGGDTQAAALTGDKYFGFLLALLAIFGVSFEVPLVIGMLNIVGILPYDAIKDKRRMIIMILFVFAAFMTPGQDPFTMLVLALSLTVLVELALQFCRFNDKRRDKKRPEWLDGDDLSASPLDTSAGGEDAPSPVETPEAVEPSRMLNPSGEASISYKPGRADFGDVL

SEQ ID NO: 21 - DNA, 945 bp, synthetic construct
  misc_feature 1..945: note = gene coding TatC P107S/G108A variant, wherein the TatC is derived from Corynebactrium glutamicum ATCC13032
  source 1..945: mol_type = other DNA
atgtccattgttgagcacatcaaagagtttcgacgccgacttcttatcgctctggcgggcatcctcgtgggcaccattatcggctttatttggtacgatttctcattttggcagatccccactttgggcgagctgctgagggatccgtactgttctctgcctgctgaatcccgctgggccatgagcgactcagaggaatgtcgactgctcgcaaccggcccgtttgatccattcatgcttcgccttaaagtagcggcgttggtgggtatggttcttggctcacccgtgtggctgagccagctgtggggctttatcacctccgcattgatgaagaatgagcgccgttacaccgcaatcttcgtcacgattgctgttgtgctgtttgtcggcggtgctgttcttgcgtacttcgtcgttgcatatggtttggagttcctccttaccattggtggagacacccaggcagcggccctgactggtgataagtacttcggattcttgctcgcgttgttggcgattttcggcgtgagcttcgaagttccactggtgatcggcatgctcaacattgtgggtatcttgccttacgatgccattaaagataagcgacgcatgatcatcatgattttgttcgtgttcgctgctttcatgacacccggccaggatcctttcaccatgttggtgttggcgctttcactcaccgttctggtagagcttgccctgcagttctgtcgtttcaacgacaaacgccgggacaagaagcgcccagaatggcttgatggcgatgacctctctgcatcaccactggatacttctgctggtggagaagatgctccaagcccagtcgaaaccccagaggcggtggagccttcgcggatgctgaacccaagtggggaggcgtcgataagctataaacccgggcgcgccgacttcggtgacgtgctctaa

SEQ ID NO: 22 - protein, 314 aa, synthetic construct
  REGION 1..314: note = TatC T106A/G108A variant, wherein the TatC is derived from Corynebactrium glutamicum ATCC13032
MSIVEHIKEFRRRLLIALAGILVGTIIGFIWYDFSFWQIPTLGELLRDPYCSLPAESRWAMSDSEECRLLATGPFDPFMLRLKVAALVGMVLGSPVWLSQLWGFIAPALMKNERRYTAIFVTIAVVLFVGGAVLAYFVVAYGLEFLLTIGGDTQAAALTGDKYFGFLLALLAIFGVSFEVPLVIGMLNIVGILPYDAIKDKRRMIIMILFVFAAFMTPGQDPFTMLVLALSLTVLVELALQFCRFNDKRRDKKRPEWLDGDDLSASPLDTSAGGEDAPSPVETPEAVEPSRMLNPSGEASISYKPGRADFGDVL

SEQ ID NO: 23 - DNA, 945 bp, synthetic construct
  misc_feature 1..945: note = gene coding TatC T106A/G108A variant, wherein the TatC is derived from Corynebactrium glutamicum ATCC13032
  source 1..945: mol_type = other DNA
atgtccattgttgagcacatcaaagagtttcgacgccgacttcttatcgctctggcgggcatcctcgtgggcaccattatcggctttatttggtacgatttctcattttggcagatccccactttgggcgagctgctgagggatccgtactgttctctgcctgctgaatcccgctgggccatgagcgactcagaggaatgtcgactgctcgcaaccggcccgtttgatccattcatgcttcgccttaaagtagcggcgttggtgggtatggttcttggctcacccgtgtggctgagccagctgtggggctttatcgcaccagcattgatgaagaatgagcgccgttacaccgcaatcttcgtcacgattgctgttgtgctgtttgtcggcggtgctgttcttgcgtacttcgtcgttgcatatggtttggagttcctccttaccattggtggagacacccaggcagcggccctgactggtgataagtacttcggattcttgctcgcgttgttggcgattttcggcgtgagcttcgaagttccactggtgatcggcatgctcaacattgtgggtatcttgccttacgatgccattaaagataagcgacgcatgatcatcatgattttgttcgtgttcgctgctttcatgacacccggccaggatcctttcaccatgttggtgttggcgctttcactcaccgttctggtagagcttgccctgcagttctgtcgtttcaacgacaaacgccgggacaagaagcgcccagaatggcttgatggcgatgacctctctgcatcaccactggatacttctgctggtggagaagatgctccaagcccagtcgaaaccccagaggcggtggagccttcgcggatgctgaacccaagtggggaggcgtcgataagctataaacccgggcgcgccgacttcggtgacgtgctctaa

SEQ ID NO: 24 - protein, 314 aa, synthetic construct
  REGION 1..314: note = TatC T106A/P107S/G108A variant, wherein the TatC is derived from Corynebactrium glutamicum ATCC13032
MSIVEHIKEFRRRLLIALAGILVGTIIGFIWYDFSFWQIPTLGELLRDPYCSLPAESRWAMSDSEECRLLATGPFDPFMLRLKVAALVGMVLGSPVWLSQLWGFIASALMKNERRYTAIFVTIAVVLFVGGAVLAYFVVAYGLEFLLTIGGDTQAAALTGDKYFGFLLALLAIFGVSFEVPLVIGMLNIVGILPYDAIKDKRRMIIMILFVFAAFMTPGQDPFTMLVLALSLTVLVELALQFCRFNDKRRDKKRPEWLDGDDLSASPLDTSAGGEDAPSPVETPEAVEPSRMLNPSGEASISYKPGRADFGDVL

SEQ ID NO: 25 - DNA, 945 bp, synthetic construct
  misc_feature 1..945: note = gene coding TatC T106A/P107S/G108A variant, wherein the TatC is derived from Corynebactrium glutamicum ATCC13032
  source 1..945: mol_type = other DNA
atgtccattgttgagcacatcaaagagtttcgacgccgacttcttatcgctctggcgggcatcctcgtgggcaccattatcggctttatttggtacgatttctcattttggcagatccccactttgggcgagctgctgagggatccgtactgttctctgcctgctgaatcccgctgggccatgagcgactcagaggaatgtcgactgctcgcaaccggcccgtttgatccattcatgcttcgccttaaagtagcggcgttggtgggtatggttcttggctcacccgtgtggctgagccagctgtggggctttatcgcatccgcattgatgaagaatgagcgccgttacaccgcaatcttcgtcacgattgctgttgtgctgtttgtcggcggtgctgttcttgcgtacttcgtcgttgcatatggtttggagttcctccttaccattggtggagacacccaggcagcggccctgactggtgataagtacttcggattcttgctcgcgttgttggcgattttcggcgtgagcttcgaagttccactggtgatcggcatgctcaacattgtgggtatcttgccttacgatgccattaaagataagcgacgcatgatcatcatgattttgttcgtgttcgctgctttcatgacacccggccaggatcctttcaccatgttggtgttggcgctttcactcaccgttctggtagagcttgccctgcagttctgtcgtttcaacgacaaacgccgggacaagaagcgcccagaatggcttgatggcgatgacctctctgcatcaccactggatacttctgctggtggagaagatgctccaagcccagtcgaaaccccagaggcggtggagccttcgcggatgctgaacccaagtggggaggcgtcgataagctataaacccgggcgcgccgacttcggtgacgtgctctaa

SEQ ID NO: 26 - protein, 254 aa, synthetic construct
  REGION 1..254: note = TatC protein derived from Bacillus subtilis subsp. subtilis (WP_010886426.1)
MTRMKVNQMSLLEHIAELRKRLLIVALAFVVFFIAGFFLAKPIIVYLQETDEAKQLTLNAFNLTDPLYVFMQFAFIIGIVLTSPVILYQLWAFVSPGLYEKERKVTLSYIPVSILLFLAGLSFSYYILFPFVVDFMKRISQDLNVNQVIGINEYFHFLLQLTIPFGLLFQMPVILMFLTRLGIVTPMFLAKIRKYAYFTLLVIAALITPPELLSHMMVTVPLLILYEISILISKAAYRKAQKSSAADRDVSSGQ

SEQ ID NO: 27 - DNA, 765 bp, synthetic construct
  misc_feature 1..765: note = gene coding TatC protein derived from Bacillus subtilis subsp. subtilis
  source 1..765: mol_type = other DNA
atgacacgaatgaaagtgaatcaaatgtcgctgctggagcatattgctgagcttcgaaaacggttgctgattgtagcgctggcgtttgtcgttttctttattgctggattttttttagcaaagccgattattgtgtatctgcaagaaacagatgaagcgaagcagcttacgcttaacgcgtttaacctgacagacccgctttatgtgtttatgcaatttgcgtttatcatcggcatagtcttgacctcgccggttattctttatcagctttgggcttttgtgagcccgggcctctatgagaaagagcgcaaagtaacgctcagctacattccggtctctattttgctgtttttagcgggcttatctttttcatattatattttatttccttttgttgttgattttatgaagcggatttctcaggacttgaatgtcaatcaggtgatcggaattaatgaatattttcattttcttctgcagctgacgattccgtttggactgctgttccaaatgccggtcatcctcatgtttttgacaaggctcggaattgtgacaccgatgttcttggcgaaaatcagaaagtatgcgtattttacgctgctggtgatcgcagccctgattacaccgcctgagcttctgtcccatatgatggtcacagtcccgcttttgattttatatgaaatcagtatccttatatcgaaggccgcttatcggaaagcacagaaaagcagtgctgccgatcgggacgtgtcttctgggcaataa

SEQ ID NO: 28 - protein, 258 aa, synthetic construct
  REGION 1..258: note = TatC P97S variant, wherein the TatC is derived from Escherichia coli K-12
MSVEDTQPLITHLIELRKRLLNCIIAVIVIFLCLVYFANDIYHLVSAPLIKQLPQGSTMIATDVASPFFTPIKLTFMVSLILSAPVILYQVWAFIASALYKHERRLVVPLLVSSSLLFYIGMAFAYFVVFPLAFGFLANTAPEGVQVSTDIASYLSFVMALFMAFGVSFEVPVAIVLLCWMGITSPEDLRKKRPYVLVGAFVVGMLLTPPDVFSQTLLAIPMYCLFEIGVFFSRFYVGKGRNREEENDAEAESEKTEE

SEQ ID NO: 29 - DNA, 777 bp, synthetic construct
  misc_feature 1..777: note = gene coding TatC P97S variant, wherein the TatC is derived from Escherichia coli K-12
  source 1..777: mol_type = other DNA
atgtctgtagaagatactcaaccgcttatcacgcatctgattgagctgcgtaagcgtctgctgaactgcattatcgcggtgatcgtgatattcctgtgtctggtctatttcgccaatgacatctatcacctggtatccgcgccattgatcaagcagttgccgcaaggttcaacgatgatcgccaccgacgtggcctcgccgttctttacgccgatcaagctgacctttatggtgtcgctgattctgtcagcgccggtgattctctatcaggtgtgggcatttatcgcctccgcgctgtataagcatgaacgtcgcctggtggtgccgctgctggtttccagctctctgctgttttatatcggcatggcattcgcctactttgtggtctttccgctggcatttggcttccttgccaataccgcgccggaaggggtgcaggtatccaccgacatcgccagctatttaagcttcgttatggcgctgtttatggcgtttggtgtctcctttgaagtgccggtagcaattgtgctgctgtgctggatggggattacctcgccagaagacttacgcaaaaaacgcccgtatgtgctggttggtgcattcgttgtcgggatgttgctgacgccgccggatgtcttctcgcaaacgctgttggcgatcccgatgtactgtctgtttgaaatcggtgtcttcttctcacgcttttacgttggtaaagggcgaaatcgggaagaggaaaacgacgctgaagcagaaagcgaaaaaactgaagaataa

SEQ ID NO: 30 - protein, 254 aa, synthetic construct
  REGION 1..254: note = TatC S95A/P96S/G97A variant, wherein the TatC is derived from Bacillus subtilis subsp. subtilis
MTRMKVNQMSLLEHIAELRKRLLIVALAFVVFFIAGFFLAKPIIVYLQETDEAKQLTLNAFNLTDPLYVFMQFAFIIGIVLTSPVILYQLWAFVASALYEKERKVTLSYIPVSILLFLAGLSFSYYILFPFVVDFMKRISQDLNVNQVIGINEYFHFLLQLTIPFGLLFQMPVILMFLTRLGIVTPMFLAKIRKYAYFTLLVIAALITPPELLSHMMVTVPLLILYEISILISKAAYRKAQKSSAADRDVSSGQ

SEQ ID NO: 31 - DNA, 765 bp, synthetic construct
  misc_feature 1..765: note = gene coding TatC S95A/P96S/G97A variant, wherein the TatC is derived from Bacillus subtilis subsp. subtilis
  source 1..765: mol_type = other DNA
atgacacgaatgaaagtgaatcaaatgtcgctgctggagcatattgctgagcttcgaaaacggttgctgattgtagcgctggcgtttgtcgttttctttattgctggattttttttagcaaagccgattattgtgtatctgcaagaaacagatgaagcgaagcagcttacgcttaacgcgtttaacctgacagacccgctttatgtgtttatgcaatttgcgtttatcatcggcatagtcttgacctcgccggttattctttatcagctttgggcttttgtggcatccgcactctatgagaaagagcgcaaagtaacgctcagctacattccggtctctattttgctgtttttagcgggcttatctttttcatattatattttatttccttttgttgttgattttatgaagcggatttctcaggacttgaatgtcaatcaggtgatcggaattaatgaatattttcattttcttctgcagctgacgattccgtttggactgctgttccaaatgccggtcatcctcatgtttttgacaaggctcggaattgtgacaccgatgttcttggcgaaaatcagaaagtatgcgtattttacgctgctggtgatcgcagccctgattacaccgcctgagcttctgtcccatatgatggtcacagtcccgcttttgattttatatgaaatcagtatccttatatcgaaggccgcttatcggaaagcacagaaaagcagtgctgccgatcgggacgtgtcttctgggcaataa

SEQ ID NO: 32 - protein, 106 aa, synthetic construct
  REGION 1..106: note = bCOL6_2 polypeptide
GSRGEKGSRGPKGYKGEKGKRGMDGVDGMKGETGFPGLPGCKGSPGFDGIQGPPGPKGDPGAFGLKGQKGEPGADGEPGRPGSTGPPGDEGEPGEPGPPGHHHHHH

SEQ ID NO: 33 - DNA, 321 bp, synthetic construct
  misc_feature 1..321: note = gene coding bCOL6_2 polypeptide
  source 1..321: mol_type = other DNA
ggcagccgcggagaaaaaggctcgagaggccccaaggggtacaaaggagagaaaggcaagcgcggaatggacggcgttgatgggatgaaaggggaaactggctttccaggccttccagggtgtaaaggctcccccgggtttgatggcatacagggcccaccggggcccaaaggcgatcctggtgcctttggacttaagggtcaaaagggagaaccgggggccgatggtgaaccgggtcgccccgggagtactgggcctccaggagatgaaggcgaaccaggtgagcccgggccccctggtcatcaccatcaccatcactaa

SEQ ID NO: 34 - protein, 16 aa, synthetic construct
  REGION 1..16: note = YGK peptide
YGKPVAVPARHHHHHH

SEQ ID NO: 35 - DNA, 51 bp, synthetic construct
  misc_feature 1..51: note = gene coding YGK peptide
  source 1..51: mol_type = other DNA
tacggaaagccagtcgcagttcccgcaagacatcaccatcaccatcactaa

SEQ ID NO: 36 - DNA, 44 bp, synthetic construct
  misc_feature 1..44: note = primer_bCOL6_1_F
  source 1..44: mol_type = other DNA
ggccaacgcccttggagcaggtggacctggtgaacggggcccac

SEQ ID NO: 37 - DNA, 47 bp, synthetic construct
  misc_feature 1..47: note = primer_bCOL6_1_R
  source 1..47: mol_type = other DNA
aacacgatctagattagtgatggtgatggtgatgaaagccaggaaag

SEQ ID NO: 38 - DNA, 36 bp, synthetic construct
  misc_feature 1..36: note = primer_TatC_F
  source 1..36: mol_type = other DNA
taggcttatgggcatgtccattgttgagcacatcaa

SEQ ID NO: 39 - DNA, 36 bp, synthetic construct
  misc_feature 1..36: note = primer_TatC_R
  source 1..36: mol_type = other DNA
cagcggccgcaactagtttagagcacgtcaccgaag

SEQ ID NO: 40 - DNA, 32 bp, synthetic construct
  misc_feature 1..32: note = primer_CgR0949_F
  source 1..32: mol_type = other DNA
aaaggaaacactatgcaaataaaccgccgagg

SEQ ID NO: 41 - DNA, 18 bp, synthetic construct
  misc_feature 1..18: note = primer_CgR0949_R
  source 1..18: mol_type = other DNA
tgctccaagggcgttggc

SEQ ID NO: 42 - DNA, 40 bp, synthetic construct
  misc_feature 1..40: note = primer_Pcj7_F
  source 1..40: mol_type = other DNA
gggaacaaaagctggatatcagaaacatcccagcgctact

SEQ ID NO: 43 - DNA, 34 bp, synthetic construct
  misc_feature 1..34: note = primer_Pcj7_R
  source 1..34: mol_type = other DNA
gtttatttgcatagtgtttcctttcgttgggtac

SEQ ID NO: 44 - DNA, 43 bp, synthetic construct
  misc_feature 1..43: note = primer_Ppyk_F
  source 1..43: mol_type = other DNA
atcaccatcactaatctagatcgtgttcttcctgttgaagaag

SEQ ID NO: 45 - DNA, 31 bp, synthetic construct
  misc_feature 1..31: note = primer_Ppyk_R
  source 1..31: mol_type = other DNA
caacaatggacatgcccataagcctagtacg

SEQ ID NO: 46 - DNA, 27 bp, synthetic construct
  misc_feature 1..27: note = primer_T106A_R
  source 1..27: mol_type = other DNA
cttcatcaaacctggtgcgataaagcc

SEQ ID NO: 47 - DNA, 25 bp, synthetic construct
  misc_feature 1..25: note = primer_T106A_F
  source 1..25: mol_type = other DNA
atcgcaccaggtttgatgaagaatg

SEQ ID NO: 48 - DNA, 27 bp, synthetic construct
  misc_feature 1..27: note = primer_P107S_R
  source 1..27: mol_type = other DNA
cttcatcaaaccggaggtgataaagcc

SEQ ID NO: 49 - DNA, 25 bp, synthetic construct
  misc_feature 1..25: note = primer_P107S_F
  source 1..25: mol_type = other DNA
atcacctccggtttgatgaagaatg

SEQ ID NO: 50 - DNA, 27 bp, synthetic construct
  misc_feature 1..27: note = primer_G108A_R
  source 1..27: mol_type = other DNA
cttcatcaatgctggggtgataaagcc

SEQ ID NO: 51 - DNA, 25 bp, synthetic construct
  misc_feature 1..25: note = primer_G108A_F
  source 1..25: mol_type = other DNA
atcaccccagcattgatgaagaatg

SEQ ID NO: 52 - DNA, 27 bp, synthetic construct
  misc_feature 1..27: note = primer_T106A_P107S_R
  source 1..27: mol_type = other DNA
cttcatcaaaccggatgcgataaagcc

SEQ ID NO: 53 - DNA, 25 bp, synthetic construct
  misc_feature 1..25: note = primer_T106A_P107S_F
  source 1..25: mol_type = other DNA
atcgcatccggtttgatgaagaatg

SEQ ID NO: 54 - DNA, 27 bp, synthetic construct
  misc_feature 1..27: note = primer_P107S_G108A_R
  source 1..27: mol_type = other DNA
cttcatcaatgcggaggtgataaagcc

SEQ ID NO: 55 - DNA, 25 bp, synthetic construct
  misc_feature 1..25: note = primer_P107S_G108A_F
  source 1..25: mol_type = other DNA
atcacctccgcattgatgaagaatg

SEQ ID NO: 56 - DNA, 27 bp, synthetic construct
  misc_feature 1..27: note = primer_T106A_G108A_R
  source 1..27: mol_type = other DNA
cttcatcaatgctggtgcgataaagcc

SEQ ID NO: 57 - DNA, 25 bp, synthetic construct
  misc_feature 1..25: note = primer_T106A_G108A_F
  source 1..25: mol_type = other DNA
atcgcaccagcattgatgaagaatg

SEQ ID NO: 58 - DNA, 27 bp, synthetic construct
  misc_feature 1..27: note = primer_T106A_P107S_G108A_R
  source 1..27: mol_type = other DNA
cttcatcaatgcggatgcgataaagcc

SEQ ID NO: 59 - DNA, 25 bp, synthetic construct
  misc_feature 1..25: note = primer_T106A_P107S_G108A_F
  source 1..25: mol_type = other DNA
atcgcatccgcattgatgaagaatg

SEQ ID NO: 60 - DNA, 32 bp, synthetic construct
  misc_feature 1..32: note = primer_EcTatC_F
  source 1..32: mol_type = other DNA
taggcttatgggcatgtctgtagaagatactc

SEQ ID NO: 61 - DNA, 37 bp, synthetic construct
  misc_feature 1..37: note = primer_EcTatC_R
  source 1..37: mol_type = other DNA
cagcggccgcaactagtttattcttcagttttttcgc

SEQ ID NO: 62 - DNA, 30 bp, synthetic construct
  misc_feature 1..30: note = primer_EcTatC_mut_R
  source 1..30: mol_type = other DNA
gcttatacagcgcggaggcgataaatgccc

SEQ ID NO: 63 - DNA, 30 bp, synthetic construct
  misc_feature 1..30: note = primer_EcTatC_mut_F
  source 1..30: mol_type = other DNA
gggcatttatcgcctccgcgctgtataagc

SEQ ID NO: 64 - DNA, 31 bp, synthetic construct
  misc_feature 1..31: note = primer_BsTatC_F
  source 1..31: mol_type = other DNA
taggcttatgggcatgacacgaatgaaagtg

SEQ ID NO: 65 - DNA, 36 bp, synthetic construct
  misc_feature 1..36: note = primer_BsTatC_R
  source 1..36: mol_type = other DNA
cagcggccgcaactagtttattgcccagaagacacg

SEQ ID NO: 66 - DNA, 33 bp, synthetic construct
  misc_feature 1..33: note = primer_BsTatC_mut_R
  source 1..33: mol_type = other DNA
ctttctcatagagtgcggatgccacaaaagccc

SEQ ID NO: 67 - DNA, 33 bp, synthetic construct
  misc_feature 1..33: note = primer_BsTatC_mut_F
  source 1..33: mol_type = other DNA
gggcttttgtggcatccgcactctatgagaaag

SEQ ID NO: 68 - DNA, 39 bp, synthetic construct
  misc_feature 1..39: note = primer_pDZ_tatC_F
  source 1..39: mol_type = other DNA
cggtacccggggatccatgtccattgttgagcacatcaa

SEQ ID NO: 69 - DNA, 38 bp, synthetic construct
  misc_feature 1..38: note = primer_pDZ_tatC_R
  source 1..38: mol_type = other DNA
cctgcaggtcgactctagattagagcacgtcaccgaag

SEQ ID NO: 70 - DNA, 49 bp, synthetic construct
  misc_feature 1..49: note = primer_bCOL6_1_R2
  source 1..49: mol_type = other DNA
gcggccgcaactagtttagtgatggtgatggtgatgaaagccaggaaag

SEQ ID NO: 71 - DNA, 38 bp, synthetic construct
  misc_feature 1..38: note = primer_bCOL6_2_F
  source 1..38: mol_type = other DNA
ggccaacgcccttggagcaggcagccgcggagaaaaag

SEQ ID NO: 72 - DNA, 44 bp, synthetic construct
  misc_feature 1..44: note = primer_bCOL6_2_R
  source 1..44: mol_type = other DNA
gcggccgcaactagtttagtgatggtgatggtgatgaccagggg

SEQ ID NO: 73 - DNA, 35 bp, synthetic construct
  misc_feature 1..35: note = primer_YGK_F
  source 1..35: mol_type = other DNA
ggccaacgcccttggagcatatcataagcctgtgg

SEQ ID NO: 74 - DNA, 44 bp, synthetic construct
  misc_feature 1..44: note = primer_YGK_R
  source 1..44: mol_type = other DNA
gcggccgcaactagtttagtgatggtgatggtgatgtcttgcgg

SEQ ID NO: 75 - protein, 6 aa, synthetic construct
  REGION 1..6: note = His tag
HHHHHH